European Patent Specification EP 3 790 984 B1, published November 22, 2023. Title: METHODS FOR EARLY PREDICTION, TREATMENT RESPONSE, RECURRENCE AND PROGNOSIS MONITORING OF BREAST CANCER. Applicant: TAIPEI MEDICAL UNIVERSITY LIN, RUO-KAI HUNG, CHIN-SHENG WANG, SHENG-CHAO CHUNG, YU-MEI SU, CHIH-MING. The sequence listing filed with the application follows.

SEQUENCE LISTING (19 sequences)

SEQ ID NO: 1 - DNA, 26 bp, artificial sequence
  synthetic polynucleotide
gttttttatttttgtcgttgcgtttc

SEQ ID NO: 2 - DNA, 20 bp, artificial sequence
  synthetic polynucleotide
cgaaaaaaattccccgacct

SEQ ID NO: 3 - DNA, 25 bp, artificial sequence
  synthetic polynucleotide
gtagttgttttcggttttcggtttc

SEQ ID NO: 4 - DNA, 26 bp, artificial sequence
  synthetic polynucleotide
tactatcgccgaccttattaaaaacg

SEQ ID NO: 5 - DNA, 20 bp, artificial sequence
  synthetic polynucleotide
gagatagggcggagtttttc

SEQ ID NO: 6 - DNA, 22 bp, artificial sequence
  synthetic polynucleotide
cttaaccgcgatactaaacgtt

SEQ ID NO: 7 - DNA, 25 bp, artificial sequence
  synthetic polynucleotide
gagtgtagttgatagtaggtacggc

SEQ ID NO: 8 - DNA, 30 bp, artificial sequence
  synthetic polynucleotide
gtaaatttactaaaaaaataaaaaaaccgt

SEQ ID NO: 9 - DNA, 25 bp, artificial sequence
  synthetic polynucleotide
ttttattggtttttcgtaagtatcg

SEQ ID NO: 10 - DNA, 25 bp, artificial sequence
  synthetic polynucleotide
cataacaacaacgtacctctacgtc

SEQ ID NO: 11 - DNA, 20 bp, artificial sequence
  synthetic polynucleotide
tttagttgttggtcggaagc

SEQ ID NO: 12 - DNA, 21 bp, artificial sequence
  synthetic polynucleotide
cgacctcactaataaaacgca

SEQ ID NO: 13 - DNA, 25 bp, artificial sequence
  synthetic polynucleotide
tgtcgcgttggtttttcgttcgttt

SEQ ID NO: 14 - DNA, 26 bp, artificial sequence
  synthetic polynucleotide
ctaaaacaacccattacgaaaaacgc

SEQ ID NO: 15 - DNA, 24 bp, artificial sequence
  synthetic polynucleotide
ggtcgatgttgtcgttcgggtgga

SEQ ID NO: 16 - DNA, 26 bp, artificial sequence
  synthetic polynucleotide
agggaggtcgagtagcggagagtgtg

SEQ ID NO: 17 - DNA, 23 bp, artificial sequence
  synthetic polynucleotide
tcgggaggggtcggtggtttgag

SEQ ID NO: 18 - DNA, 24 bp, artificial sequence
  synthetic polynucleotide
gaagtgggcgttcgtcgtttcgtt

SEQ ID NO: 19 - DNA, 149 bp, artificial sequence
  synthetic polynucleotide
cgcaggccaggccctctattcctgtcgctgcgccccgccttgccggctgcgtgtcacccccccccctgccgcgctggctccccgtccgtcccaccagccttgctgtcctgggcaggccggggaattcctcccggttcctggaaaaaaca